European Patent Application EP 4 389 771 A1, published June 26, 2024. Title: 包含抗TIGIT抗体和TGF-βR的融合蛋白、其药物组合物及用途. Applicant: 中山康方生物医药有限公司. The sequence listing filed with the application follows.

SEQUENCE LISTING (48 sequences)

SEQ ID NO: 1 - protein, 121 aa, synthetic construct
  source 1..121: note = 26B12VH
EVQLQESGPGLVKPSQSLSLTCTVTGHSFTSDYAWNWIRQFPGNRLEWMGYISYSDSTNYNPSLKSRISITRDTSKNQFFLQMNSVTTEDTATYYCARLDYGNYGGAMDYWGQGTSVTVSS

SEQ ID NO: 2 - DNA, 363 bp, synthetic construct
  source 1..363: mol_type = other DNA; note = 26B12VH
gaggtgcagctgcaggagtctggacctggcctggtgaaaccctctcagtctctgtccctcacctgcactgtcactggccactcattcaccagtgattatgcctggaactggatccggcagtttccaggaaacagactggagtggatgggctacataagctacagtgatagcactaactacaacccatctctcaaaagtcgaatctctatcactcgagacacatccaagaaccagttcttcttgcagatgaattctgtgactactgaggacacagccacatattactgtgcaagattggactatggtaactacggtggggctatggactactggggtcaagggacctcagtcaccgtctcctca

SEQ ID NO: 3 - protein, 9 aa, synthetic construct
  source 1..9: note = HCDR1
GHSFTSDYA

SEQ ID NO: 4 - protein, 7 aa, synthetic construct
  source 1..7: note = HCDR2
ISYSDST

SEQ ID NO: 5 - protein, 14 aa, synthetic construct
  source 1..14: note = HCDR3
ARLDYGNYGGAMDY

SEQ ID NO: 6 - protein, 107 aa, synthetic construct
  source 1..107: note = 26B12VL
DIVLTQSHEFMSTSLRDRVSITCKSSQHVSTAVAWYQQKPGQSPKLLIYSASYRYTGVPDRFTGSGSGTDFTFTISSVKAEDLAVYYCQQHYITPWTFGGGTKLEIK

SEQ ID NO: 7 - DNA, 321 bp
gatattgtgctaactcagtctcacgaattcatgtccacctcattacgagacagggtcagcatcacctgcaaatccagtcaacatgtgagtactgctgtagcctggtatcaacagaaaccaggacaatctcctaaactactgatttactcggcatcctaccggtacactggagtccctgatcgcttcactggcagtggatctgggacggatttcactttcaccatcagcagtgtgaaggctgaagacctggcagtttattactgtcagcaacattatattactccgtggacgttcggtggaggcaccaagctggaaataaaa

SEQ ID NO: 8 - protein, 6 aa, synthetic construct
  source 1..6: note = LCDR1
QHVSTA

SEQ ID NO: 9 - skipped

SEQ ID NO: 10 - protein, 9 aa, synthetic construct
  source 1..9: note = LCDR3
QQHYITPWT

SEQ ID NO: 11 - protein, 121 aa, synthetic construct
  source 1..121: note = 26B12H1VH
DVQLQESGPGLVKPSQTLSLTCTVSGHSFTSDYAWNWIRQFPGKGLEWIGYISYSDSTNYNPSLKSRITISRDTSKNQFFLQLNSVTAADTATYYCARLDYGNYGGAMDYWGQGTSVTVSS

SEQ ID NO: 12 - DNA, 363 bp, synthetic construct
  source 1..363: mol_type = other DNA; note = 26B12H1VH
gatgtgcagctgcaggagagcggccccggactggtgaagccttcccagaccctgtctctgacctgtacagtgtctggccacagcttcacatccgactacgcctggaactggatcaggcagtttccaggcaagggcctggagtggatcggctacatctcttatagcgactccaccaactataatccctctctgaagagccggatcaccatcagcagagatacatccaagaaccagttctttctgcagctgaacagcgtgacagccgccgacaccgccacatactattgcgcccggctggactacggcaattatggcggagccatggattactggggccagggcacctccgtgacagtgagctcc

SEQ ID NO: 13 - protein, 121 aa, synthetic construct
  source 1..121: note = 26B12H2VH
DVQLQESGPGLVKPSQTLSLTCTVSGHSFTSDYAWSWIRQPPGKGLEWIGYISYSDSTNYNPSLKSRVTISRDTSKNQFSLKLSSVTAADTAVYYCARLDYGNYGGAMDYWGQGTSVTVSS

SEQ ID NO: 14 - DNA, 363 bp, synthetic construct
  source 1..363: mol_type = other DNA; note = 26B12H2VH
gatgtgcagctgcaggagtctggcccaggactggtgaagccaagccagaccctgtccctgacctgtacagtgtccggccactcttttacaagcgactacgcctggtcttggatcaggcagccccctggcaagggactggagtggatcggctacatctcctattctgacagcaccaactataatccctccctgaagtctcgggtgaccatctctagagatacaagcaagaaccagttctccctgaagctgagctccgtgaccgcagcagacacagccgtgtactattgcgcccggctggactacggcaattatggcggagccatggattactggggccagggcaccagcgtgacagtgtctagc

SEQ ID NO: 15 - protein, 121 aa, synthetic construct
  source 1..121: note = 26B12H3VH
DVQLQESGPGLVKPSQTLSLTCTVSGHSFTSDYAWSWIRQPPGKGLEWIGYISYSDSTNYNPSLKSRVTISVDTSKNQFSLKLSSVTAADTAVYYCARLDYGNYGGAMDYWGQGTSVTVSS

SEQ ID NO: 16 - DNA, 363 bp, synthetic construct
  source 1..363: mol_type = other DNA; note = 26B12H3VH
gatgtgcagctgcaggagtctggcccaggactggtgaagccaagccagaccctgtccctgacctgtacagtgtccggccactcttttacaagcgactacgcctggtcttggatcagacagccccctggcaagggactggagtggatcggctacatctcctattctgacagcaccaactataatccctccctgaagtctagagtgaccatctctgtggatacaagcaagaaccagttctccctgaagctgagctccgtgaccgcagcagacacagccgtgtactattgcgcccggctggactacggcaattatggcggagccatggattactggggccagggcaccagcgtgacagtgtctagc

SEQ ID NO: 17 - protein, 121 aa, synthetic construct
  source 1..121: note = 26B12H4VH
DVQLQESGPGLVKPSQTLSLTCTVSGHSFTSDYAWNWIRQFPGKGLEWMGYISYSDSTNYNPSLKSRITISRDTSKNQFFLQLNSVTAADTATYYCARLDYGNYGGAMDYWGQGTSVTVSS

SEQ ID NO: 18 - DNA, 363 bp, synthetic construct
  source 1..363: mol_type = other DNA; note = 26B12H4VH
gatgtgcagctgcaggagagcggccccggactggtgaagccttcccagaccctgtctctgacctgtacagtgtctggccacagcttcacatccgactacgcctggaactggatcaggcagtttccaggcaagggcctggagtggatgggctacatctcttatagcgactccaccaactataatccctctctgaagagccggatcaccatcagcagagatacatccaagaaccagttctttctgcagctgaacagcgtgacagccgccgacaccgccacatactattgcgcccggctggactacggcaattatggcggagccatggattactggggccagggcacctccgtgacagtgagctcc

SEQ ID NO: 19 - protein, 107 aa, synthetic construct
  source 1..107: note = 26B12L1VL
DIQMTQSPKSLSTSVGDRVTITCRSSQHVSTAVAWYQQKPGKSPKLLIYSASYRYSGVPDRFSGSGSGTDFTFTISSVQPEDFATYYCQQHYITPWTFGGGTKLEIK

SEQ ID NO: 20 - DNA, 321 bp, synthetic construct
  source 1..321: mol_type = other DNA; note = 26B12L1VL
gacatccagatgacccagtcccctaagtccctgtctacaagcgtgggcgatcgggtgaccatcacatgtagaagctcccagcacgtgtctaccgcagtggcatggtaccagcagaagccaggcaagagccctaagctgctgatctattccgcctcttacaggtattccggagtgccagaccggtttagcggctccggctctggcaccgatttcacctttacaatctctagcgtgcagccagaggacttcgccacatactattgccagcagcactacatcaccccatggaccttcggcggcggcacaaagctggagatcaag

SEQ ID NO: 21 - protein, 107 aa, synthetic construct
  source 1..107: note = 26B12L2VL
DIQMTQSPSSLSASVGDRVTITCRSSQHVSTALAWYQQKPGKSPKLLIYSASSRYSGVPDRFSGSGSGTDFTFTISSLQPEDFATYYCQQHYITPWTFGGGTKLEIK

SEQ ID NO: 22 - DNA, 321 bp, synthetic construct
  source 1..321: mol_type = other DNA; note = 26B12L2VL
gacatccagatgacccagtcccctagctccctgtctgccagcgtgggcgatagggtgaccatcacatgtagatctagccagcacgtgtctacagccctggcatggtaccagcagaagccaggcaagagccctaagctgctgatctactccgcctcctctaggtattctggagtgccagaccggttttccggctctggcagcggcaccgatttcacctttacaatcagctccctgcagccagaggacttcgccacatactattgccagcagcactatatcaccccatggaccttcggcggcggcaccaagctggagatcaag

SEQ ID NO: 23 - protein, 107 aa, synthetic construct
  source 1..107: note = 26B12L3VL
DIQMTQSPSSLSASVGDRVTITCRASQHVSTALAWYQQKPGKAPKLLIYSASSLQSGVPSRFSGSGSGTDFTLTISSLQPEDFATYYCQQHYITPWTFGGGTKLEIK

SEQ ID NO: 24 - DNA, 321 bp, synthetic construct
  source 1..321: mol_type = other DNA; note = 26B12L3VL
gacatccagatgacccagtcccctagctccctgagcgcctccgtgggcgatagggtgaccatcacatgtagagcctctcagcacgtgagcacagccctggcatggtaccagcagaagccaggcaaggcccctaagctgctgatctatagcgcctctagcctgcagtccggagtgccatctcggttctctggcagcggctccggaaccgactttaccctgacaatctcctctctgcagccagaggatttcgccacatactattgccagcagcactacatcaccccatggaccttcggcggcggcaccaagctggagatcaag

SEQ ID NO: 25 - protein, 107 aa, synthetic construct
  source 1..107: note = 26B12L4VL
DIQMTQSPKSMSTSVGDRVTITCRSSQHVSTAVAWYQQKPGKSPKLLIYSASYRYSGVPDRFSGSGSGTDFTFTISSVQPEDFATYYCQQHYITPWTFGGGTKLEIK

SEQ ID NO: 26 - DNA, 321 bp, synthetic construct
  source 1..321: mol_type = other DNA; note = 26B12L4VL
gacatccagatgacccagtcccctaagtccatgtctacaagcgtgggcgacagggtgaccatcacatgtagaagctcccagcacgtgtctaccgcagtggcatggtaccagcagaagccaggcaagagccctaagctgctgatctattccgcctcttacaggtattccggagtgccagaccggtttagcggctccggctctggcaccgatttcacctttacaatctctagcgtgcagccagaggacttcgccacatactattgccagcagcactacatcaccccatggaccttcggcggcggcacaaagctggagatcaag

SEQ ID NO: 27 - protein, 447 aa, synthetic construct
  source 1..447: note = 26B12H2L2(hG4DM)
DVQLQESGPGLVKPSQTLSLTCTVSGHSFTSDYAWSWIRQPPGKGLEWIGYISYSDSTNYNPSLKSRVTISRDTSKNQFSLKLSSVTAADTAVYYCARLDYGNYGGAMDYWGQGTSVTVSSASTKGPSVFPLAPCSRSTSESTAALGCLVKDYFPEPVTVSWNSGALTSGVHTFPAVLQSSGLYSLSSVVTVPSSSLGTKTYTCNVDHKPSNTKVDKRVESKYGPPCPPCPAPEAAGGPSVFLFPPKPKDTLMISRTPEVTCVVVDVSQEDPEVQFNWYVDGVEVHNAKTKPREEQFNSTYRVVSVLTVLHQDWLNGKEYKCKVSNKGLPSSIEKTISKAKGQPREPQVYTLPPSQEEMTKNQVSLTCLVKGFYPSDIAVEWESNGQPENNYKTTPPVLDSDGSFFLYSRLTVDKSRWQEGNVFSCSVMHEALHNHYTQKSLSLSLG

SEQ ID NO: 28 - DNA, 1341 bp, synthetic construct
  misc_feature 1..1341: note = 26B12H2L2(hG4DM)
  source 1..1341: mol_type = other DNA; note = 26B12H2L2(hG4DM)
gatgtgcagctgcaggagtctggcccaggactggtgaagccaagccagaccctgtccctgacctgtacagtgtccggccactcttttacaagcgactacgcctggtcttggatcaggcagccccctggcaagggactggagtggatcggctacatctcctattctgacagcaccaactataatccctccctgaagtctcgggtgaccatctctagagatacaagcaagaaccagttctccctgaagctgagctccgtgaccgcagcagacacagccgtgtactattgcgcccggctggactacggcaattatggcggagccatggattactggggccagggcaccagcgtgacagtgtctagcgcctccacaaaggggccctcggtcttccccctggcgccctgctccaggagcacctccgagagcacagccgccctgggctgcctggtcaaggactacttccccgaaccggtgacggtgtcgtggaactcaggcgccctgaccagcggcgtacacaccttcccggctgtcctacagtcctcaggactctactccctcagcagcgtggtgaccgtgccctccagcagcttgggcacgaagacctacacctgcaacgtagatcacaagcccagcaacaccaaggtggacaagagagttgagtccaaatatggtcccccatgcccaccatgcccagcacctgaggccgctgggggaccatcagtcttcctgttccccccaaaacccaaggacactctcatgatctcccggacccctgaggtcacgtgcgtggtggtggacgtgagccaggaagaccccgaggtccagttcaactggtacgtggatggcgtggaggtgcataatgccaagacaaagccgcgggaggagcagttcaacagcacgtaccgtgtggtcagcgtcctcaccgtcctgcaccaggactggctgaacggcaaggagtacaagtgcaaggtctccaacaaaggcctcccgtcctccatcgagaaaaccatctccaaagccaaagggcagccccgagagccacaggtgtacaccctgcccccatcccaggaggagatgaccaagaaccaggtcagcctgacctgcctggtcaaaggcttctaccccagcgacatcgccgtggagtgggagagcaatgggcagccggagaacaactacaagaccacgcctcccgtgctggactccgacggctccttcttcctctacagcaggctaaccgtggacaagagcaggtggcaggaggggaatgtcttctcatgctccgtgatgcatgaggctctgcacaaccactacacacagaagagcctctccctgtctctgggt

SEQ ID NO: 29 - protein, 214 aa, synthetic construct
  source 1..214: note = 26B12H2L2(hG4DM)
DIQMTQSPSSLSASVGDRVTITCRSSQHVSTALAWYQQKPGKSPKLLIYSASSRYSGVPDRFSGSGSGTDFTFTISSLQPEDFATYYCQQHYITPWTFGGGTKLEIKRTVAAPSVFIFPPSDEQLKSGTASVVCLLNNFYPREAKVQWKVDNALQSGNSQESVTEQDSKDSTYSLSSTLTLSKADYEKHKVYACEVTHQGLSSPVTKSFNRGEC

SEQ ID NO: 30 - DNA, 642 bp, synthetic construct
  source 1..642: mol_type = other DNA; note = 26B12H2L2(hG4DM)
gacatccagatgacccagtcccctagctccctgtctgccagcgtgggcgatagggtgaccatcacatgtagatctagccagcacgtgtctacagccctggcatggtaccagcagaagccaggcaagagccctaagctgctgatctactccgcctcctctaggtattctggagtgccagaccggttttccggctctggcagcggcaccgatttcacctttacaatcagctccctgcagccagaggacttcgccacatactattgccagcagcactatatcaccccatggaccttcggcggcggcaccaagctggagatcaagcgtacggtggcagccccatctgtcttcatttttccccctagtgacgagcagctgaaatccggaacagcctctgtggtctgtctgctgaacaatttctaccctcgcgaagccaaggtgcagtggaaagtcgataacgctctgcagagtggcaattcacaggagagcgtgactgaacaggactccaaggattctacctatagtctgagctccactctgaccctgtccaaagcagattacgaaaagcacaaagtgtatgcctgtgaggtcacccaccaggggctgagttctccagtcaccaaatccttcaacagaggcgaatgt

SEQ ID NO: 31 - protein, 451 aa, synthetic construct
  source 1..451: note = 26B12H2L2(hG1DM)
DVQLQESGPGLVKPSQTLSLTCTVSGHSFTSDYAWSWIRQPPGKGLEWIGYISYSDSTNYNPSLKSRVTISRDTSKNQFSLKLSSVTAADTAVYYCARLDYGNYGGAMDYWGQGTSVTVSSASTKGPSVFPLAPSSKSTSGGTAALGCLVKDYFPEPVTVSWNSGALTSGVHTFPAVLQSSGLYSLSSVVTVPSSSLGTQTYICNVNHKPSNTKVDKKVEPKSCDKTHTCPPCPAPEAAGGPSVFLFPPKPKDTLMISRTPEVTCVVVDVSHEDPEVKFNWYVDGVEVHNAKTKPREEQYNSTYRVVSVLTVLHQDWLNGKEYKCKVSNKALPAPIEKTISKAKGQPREPQVYTLPPSRDELTKNQVSLTCLVKGFYPSDIAVEWESNGQPENNYKTTPPVLDSDGSFFLYSKLTVDKSRWQQGNVFSCSVMHEALHNHYTQKSLSLSPGK

SEQ ID NO: 32 - DNA, 1353 bp, synthetic construct
  misc_feature 1..1353: note = 26B12H2L2(hG1DM)
  source 1..1353: mol_type = other DNA; note = 26B12H2L2(hG1DM)
gatgtgcagctgcaggagtctggcccaggactggtgaagccaagccagaccctgtccctgacctgtacagtgtccggccactcttttacaagcgactacgcctggtcttggatcaggcagccccctggcaagggactggagtggatcggctacatctcctattctgacagcaccaactataatccctccctgaagtctcgggtgaccatctctagagatacaagcaagaaccagttctccctgaagctgagctccgtgaccgcagcagacacagccgtgtactattgcgcccggctggactacggcaattatggcggagccatggattactggggccagggcaccagcgtgacagtgtctagcgcctctaccaaggggcccagcgtgtttcctctcgccccctcctccaaaagcaccagcggaggaaccgctgctctcggatgtctggtgaaggactacttccctgaacccgtcaccgtgagctggaatagcggcgctctgacaagcggagtccatacattccctgctgtgctgcaaagcagcggactctattccctgtccagcgtcgtcacagtgcccagcagcagcctgggcacccagacctacatctgtaacgtcaaccacaagccctccaacaccaaggtggacaagaaagtggagcccaaatcctgcgacaagacacacacctgtcccccctgtcctgctcccgaagctgctggaggccctagcgtcttcctctttcctcccaaacccaaggacaccctcatgatcagcagaacccctgaagtcacctgtgtcgtcgtggatgtcagccatgaggaccccgaggtgaaattcaactggtatgtcgatggcgtcgaggtgcacaacgccaaaaccaagcccagggaggaacagtacaactccacctacagggtggtgtccgtgctgacagtcctccaccaggactggctgaacggcaaggagtacaagtgcaaggtgtccaacaaggctctccctgcccccattgagaagaccatcagcaaggccaaaggccaacccagggagccccaggtctatacactgcctccctccagggacgaactcaccaagaaccaggtgtccctgacctgcctggtcaagggcttttatcccagcgacatcgccgtcgagtgggagtccaacggacagcccgagaataactacaagaccacccctcctgtcctcgactccgacggctccttcttcctgtacagcaagctgaccgtggacaaaagcaggtggcagcagggaaacgtgttctcctgcagcgtgatgcacgaagccctccacaaccactacacccagaaaagcctgtccctgagccccggcaaa

SEQ ID NO: 33 - protein, 136 aa, synthetic construct
  source 1..136: note = TGF-RII
IPPHVQKSVNNDMIVTDNNGAVKFPQLCKFCDVRFSTCDNQKSCMSNCSITSICEKPQEVCVAVWRKNDENITLETVCHDPKLPYHDFILEDAASPKCIMKEKKKPGETFFMCSCSSDECNDNIIFSEEYNTSNPD

SEQ ID NO: 34 - protein, 503 aa, synthetic construct
  source 1..503: note = TGF-R
MEAAVAAPRPRLLLLVLAAAAAAAAALLPGATALQCFCHLCTKDNFTCVTDGLCFVSVTETTDKVIHNSMCIAEIDLIPRDRPFVCAPSSKTGSVTTTYCCNQDHCNKIELPTTVKSSPGLGPVELAAVIAGPVCFVCISLMLMVYICHNRTVIHHRVPNEEDPSLDRPFISEGTTLKDLIYDMTTSGSGSGLPLLVQRTIARTIVLQESIGKGRFGEVWRGKWRGEEVAVKIFSSREERSWFREAEIYQTVMLRHENILGFIAADNKDNGTWTQLWLVSDYHEHGSLFDYLNRYTVTVEGMIKLALSTASGLAHLHMEIVGTQGKPAIAHRDLKSKNILVKKNGTCCIADLGLAVRHDSATDTIDIAPNHRVGTKRYMAPEVLDDSINMKHFESFKRADIYAMGLVFWEIARRCSIGGIHEDYQLPYYDLVPSDPSVEEMRKVVCEQKLRPNIPNRWQSCEALRVMAKIMRECWYANGAARLTALRIKKTLSQLSQQEGIKM

SEQ ID NO: 35 - protein, 93 aa, synthetic construct
  source 1..93: note = TGF-R
LQCFCHLCTKDNFTCVTDGLCFVSVTETTDKVIHNSMCIAEIDLIPRDRPFVCAPSSKTGSVTTTYCCNQDHCNKIELPTTVKSSPGLGPVEL

SEQ ID NO: 36 - protein, 567 aa, synthetic construct
  source 1..567: note = TGF-R
MGRGLLRGLWPLHIVLWTRIASTIPPHVQKSVNNDMIVTDNNGAVKFPQLCKFCDVRFSTCDNQKSCMSNCSITSICEKPQEVCVAVWRKNDENITLETVCHDPKLPYHDFILEDAASPKCIMKEKKKPGETFFMCSCSSDECNDNIIFSEEYNTSNPDLLLVIFQVTGISLLPPLGVAISVIIIFYCYRVNRQQKLSSTWETGKTRKLMEFSEHCAIILEDDRSDISSTCANNINHNTELLPIELDTLVGKGRFAEVYKAKLKQNTSEQFETVAVKIFPYEEYASWKTEKDIFSDINLKHENILQFLTAEERKTELGKQYWLITAFHAKGNLQEYLTRHVISWEDLRKLGSSLARGIAHLHSDHTPCGRPKMPIVHRDLKSSNILVKNDLTCCLCDFGLSLRLDPTLSVDDLANSGQVGTARYMAPEVLESRMNLENVESFKQTDVYSMALVLWEMTSRCNAVGEVKDYEPPFGSKVREHPCVESMKDNVLRDRGRPEIPSFWLNHQGIQMVCETLTECWDHDPEARLTAQCVAERFSELEHLDRLSGRSCSEEKIPEDGSLNTTK

SEQ ID NO: 37 - protein, 144 aa, synthetic construct
  source 1..144: note = TGF-R
TIPPHVQKSVNNDMIVTDNNGAVKFPQLCKFCDVRFSTCDNQKSCMSNCSITSICEKPQEVCVAVWRKNDENITLETVCHDPKLPYHDFILEDAASPKCIMKEKKKPGETFFMCSCSSDECNDNIIFSEEYNTSNPDLLLVIFQ

SEQ ID NO: 38 - protein, 851 aa, synthetic construct
  source 1..851: note = TGF-R
MTSHYVIAIFALMSSCLATAGPEPGALCELSPVSASHPVQALMESFTVLSGCASRGTTGLPQEVHVLNLRTAGQGPGQLQREVTLHLNPISSVHIHHKSVVFLLNSPHPLVWHLKTERLATGVSRLFLVSEGSVVQFSSANFSLTAETEERNFPHGNEHLLNWARKEYGAVTSFTELKIARNIYIKVGEDQVFPPKCNIGKNFLSLNYLAEYLQPKAAEGCVMSSQPQNEEVHIIELITPNSNPYSAFQVDITIDIRPSQEDLEVVKNLILILKCKKSVNWVIKSFDVKGSLKIIAPNSIGFGKESERSMTMTKSIRDDIPSTQGNLVKWALDNGYSPITSYTMAPVANRFHLRLENNAEEMGDEEVHTIPPELRILLDPGALPALQNPPIRGGEGQNGGLPFPFPDISRRVWNEEGEDGLPRPKDPVIPSIQLFPGLREPEEVQGSVDIALSVKCDNEKMIVAVEKDSFQASGYSGMDVTLLDPTCKAKMNGTHFVLESPLNGCGTRPRWSALDGVVYYNSIVIQVPALGDSSGWPDGYEDLESGDNGFPGDMDEGDASLFTRPEIVVFNCSLQQVRNPSSFQEQPHGNITFNMELYNTDLFLVPSQGVFSVPENGHVYVEVSVTKAEQELGFAIQTCFISPYSNPDRMSHYTIIENICPKDESVKFYSPKRVHFPIPQADMDKKRFSFVFKPVFNTSLLFLQCELTLCTKMEKHPQKLPKCVPPDEACTSLDASIIWAMMQNKKTFTKPLAVIHHEAESKEKGPSMKEPNPISPPIFHGLDTLTVMGIAFAAFVIGALLTGALWYIYSHTGETAGRQQVPTSPPASENSSAAHSIGSTQSTPCSSSSTA

SEQ ID NO: 39 - protein, 767 aa, synthetic construct
  source 1..767: note = TGF-R
GPEPGALCELSPVSASHPVQALMESFTVLSGCASRGTTGLPQEVHVLNLRTAGQGPGQLQREVTLHLNPISSVHIHHKSVVFLLNSPHPLVWHLKTERLATGVSRLFLVSEGSVVQFSSANFSLTAETEERNFPHGNEHLLNWARKEYGAVTSFTELKIARNIYIKVGEDQVFPPKCNIGKNFLSLNYLAEYLQPKAAEGCVMSSQPQNEEVHIIELITPNSNPYSAFQVDITIDIRPSQEDLEVVKNLILILKCKKSVNWVIKSFDVKGSLKIIAPNSIGFGKESERSMTMTKSIRDDIPSTQGNLVKWALDNGYSPITSYTMAPVANRFHLRLENNAEEMGDEEVHTIPPELRILLDPGALPALQNPPIRGGEGQNGGLPFPFPDISRRVWNEEGEDGLPRPKDPVIPSIQLFPGLREPEEVQGSVDIALSVKCDNEKMIVAVEKDSFQASGYSGMDVTLLDPTCKAKMNGTHFVLESPLNGCGTRPRWSALDGVVYYNSIVIQVPALGDSSGWPDGYEDLESGDNGFPGDMDEGDASLFTRPEIVVFNCSLQQVRNPSSFQEQPHGNITFNMELYNTDLFLVPSQGVFSVPENGHVYVEVSVTKAEQELGFAIQTCFISPYSNPDRMSHYTIIENICPKDESVKFYSPKRVHFPIPQADMDKKRFSFVFKPVFNTSLLFLQCELTLCTKMEKHPQKLPKCVPPDEACTSLDASIIWAMMQNKKTFTKPLAVIHHEAESKEKGPSMKEPNPISPPIFHGLDTLTV

SEQ ID NO: 40 - protein, 456 aa, synthetic construct
  source 1..456: note = Tiragolumab
EVQLQQSGPGLVKPSQTLSLTCAISGDSVSSNSAAWNWIRQSPSRGLEWLGKTYYRFKWYSDYAVSVKGRITINPDTSKNQFSLQLNSVTPEDTAVFYCTRESTTYDLLAGPFDYWGQGTLVTVSSASTKGPSVFPLAPSSKSTSGGTAALGCLVKDYFPEPVTVSWNSGALTSGVHTFPAVLQSSGLYSLSSVVTVPSSSLGTQTYICNVNHKPSNTKVDKKVEPKSCDKTHTCPPCPAPELLGGPSVFLFPPKPKDTLMISRTPEVTCVVVDVSHEDPEVKFNWYVDGVEVHNAKTKPREEQYNSTYRVVSVLTVLHQDWLNGKEYKCKVSNKALPAPIEKTISKAKGQPREPQVYTLPPSREEMTKNQVSLTCLVKGFYPSDIAVEWESNGQPENNYKTTPPVLDSDGSFFLYSKLTVDKSRWQQGNVFSCSVMHEALHNHYTQKSLSLSPGK

SEQ ID NO: 41 - protein, 220 aa, synthetic construct
  source 1..220: note = Tiragolumab
DIVMTQSPDSLAVSLGERATINCKSSQTVLYSSNNKKYLAWYQQKPGQPPNLLIYWASTRESGVPDRFSGSGSGTDFTLTISSLQAEDVAVYYCQQYYSTPFTFGPGTKVEIKRTVAAPSVFIFPPSDEQLKSGTASVVCLLNNFYPREAKVQWKVDNALQSGNSQESVTEQDSKDSTYSLSSTLTLSKADYEKHKVYACEVTHQGLSSPVTKSFNRGEC

SEQ ID NO: 42 - protein, 126 aa, synthetic construct
  source 1..126: note = RG6058(hG4)
EVQLQQSGPGLVKPSQTLSLTCAISGDSVSSNSAAWNWIRQSPSRGLEWLGKTYYRFKWYSDYAVSVKGRITINPDTSKNQFSLQLNSVTPEDTAVFYCTRESTTYDLLAGPFDYWGQGTLVTVSS

SEQ ID NO: 43 - protein, 113 aa, synthetic construct
  source 1..113: note = RG6058(hG4)
DIVMTQSPDSLAVSLGERATINCKSSQTVLYSSNNKKYLAWYQQKPGQPPNLLIYWASTRESGVPDRFSGSGSGTDFTLTISSLQAEDVAVYYCQQYYSTPFTFGPGTKVEIK

SEQ ID NO: 44 - protein, 21 aa, synthetic construct
  source 1..21: note = linker
GGGGSGGGGSGGGGSGGGGSG

SEQ ID NO: 45 - protein, 599 aa, synthetic construct
  source 1..599: note = anti-HEL& TGFbeta
EVQLEQSGAELMKPGASVKISCKATGYTFTTYWIEWIKQRPGHSLEWIGEILPGSDSTYYNEKVKGKVTFTADASSNTAYMQLSSLTSEDSAVYYCARGDGFYVYWGQGTTLTVSSASTKGPSVFPLAPCSRSTSESTAALGCLVKDYFPEPVTVSWNSGALTSGVHTFPAVLQSSGLYSLSSVVTVPSSSLGTKTYTCNVDHKPSNTKVDKRVESKYGPPCPPCPAPEAAGGPSVFLFPPKPKDTLMISRTPEVTCVVVDVSQEDPEVQFNWYVDGVEVHNAKTKPREEQFNSTYRVVSVLTVLHQDWLNGKEYKCKVSNKGLPSSIEKTISKAKGQPREPQVYTLPPSQEEMTKNQVSLTCLVKGFYPSDIAVEWESNGQPENNYKTTPPVLDSDGSFFLYSRLTVDKSRWQEGNVFSCSVMHEALHNHYTQKSLSLSLGGGGGSGGGGSGGGGSGGGGSGIPPHVQKSVNNDMIVTDNNGAVKFPQLCKFCDVRFSTCDNQKSCMSNCSITSICEKPQEVCVAVWRKNDENITLETVCHDPKLPYHDFILEDAASPKCIMKEKKKPGETFFMCSCSSDECNDNIIFSEEYNTSNPD

SEQ ID NO: 46 - protein, 214 aa, synthetic construct
  source 1..214: note = anti-HEL& TGFbeta
DIELTQSPATLSVTPGDSVSLSCRASQSISNNLHWYQQKSHESPRLLIKYTSQSMSGIPSRFSGSGSGTDFTLSINSVETEDFGVYFCQQSGSWPRTFGGGTKLDIKRTVAAPSVFIFPPSDEQLKSGTASVVCLLNNFYPREAKVQWKVDNALQSGNSQESVTEQDSKDSTYSLSSTLTLSKADYEKHKVYACEVTHQGLSSPVTKSFNRGEC

SEQ ID NO: 47 - protein, 456 aa, synthetic construct
  source 1..456: note = RG6058(G1DM) HC
EVQLQQSGPGLVKPSQTLSLTCAISGDSVSSNSAAWNWIRQSPSRGLEWLGKTYYRFKWYSDYAVSVKGRITINPDTSKNQFSLQLNSVTPEDTAVFYCTRESTTYDLLAGPFDYWGQGTLVTVSSASTKGPSVFPLAPSSKSTSGGTAALGCLVKDYFPEPVTVSWNSGALTSGVHTFPAVLQSSGLYSLSSVVTVPSSSLGTQTYICNVNHKPSNTKVDKKVEPKSCDKTHTCPPCPAPEAAGGPSVFLFPPKPKDTLMISRTPEVTCVVVDVSHEDPEVKFNWYVDGVEVHNAKTKPREEQYNSTYRVVSVLTVLHQDWLNGKEYKCKVSNKALPAPIEKTISKAKGQPREPQVYTLPPSRDELTKNQVSLTCLVKGFYPSDIAVEWESNGQPENNYKTTPPVLDSDGSFFLYSKLTVDKSRWQQGNVFSCSVMHEALHNHYTQKSLSLSPGK

SEQ ID NO: 48 - protein, 220 aa, synthetic construct; identical to SEQ ID NO: 41
  source 1..220: note = RG6058(G1DM) LC